European Patent Application EP 4 509 494 A1, published February 19, 2025. Title: PLpro蛋白抑制剂及其制备方法和应用. Applicant: 清华大学. The sequence listing filed with the application follows.

SEQUENCE LISTING (3 sequences)

SEQ ID NO: 1 - DNA, 22 bp, synthetic construct
  source 1..22: mol_type = other DNA
ggggaacttctcctgctagaat

SEQ ID NO: 2 - DNA, 22 bp, synthetic construct
  source 1..22: mol_type = other DNA
cagacattttgctctcaagctg

SEQ ID NO: 3 - DNA, 20 bp, synthetic construct
  source 1..20: mol_type = other DNA
ttgctgctgcttgacagatt